European Patent Specification EP 3 858 852 B1, published June 21, 2023. Title: T cell receptor for identifying SSX2 antigen. Applicant: XLIFESC, LTD. Application PCT/CN2019/107097. The sequence listing filed with the application follows.

SEQUENCE LISTING (37 sequences)

SEQ ID NO: 1 - protein, 118 aa, Artificial sequence
  Synthesized polypeptide
AQTVTQSQPEMSVQEAETVTLSCTYDTSESDYYLFWYKQPPSRQMILVIRQEAYKQQNATENRFSVNFQKAAKSFSLKISDSQLGDAAMYFCAYRSGIIQGAQKLVFGQGTRLTINPN

SEQ ID NO: 2 - DNA, 354 bp, Artificial sequence
  Synthesized polynucleotide
gctcagacagtcactcagtctcaaccagagatgtctgtgcaggaggcagagaccgtgaccctgagctgcacatatgacaccagtgagagtgattattatttattctggtacaagcagcctcccagcaggcagatgattctcgttattcgccaagaagcttataagcaacagaatgcaacagagaatcgtttctctgtgaacttccagaaagcagccaaatccttcagtctcaagatctcagactcacagctgggggatgccgcgatgtatttctgtgcttataggagcggcataattcagggagcccagaagctggtatttggccaaggaaccaggctgactatcaacccaaat

SEQ ID NO: 3 - protein, 258 aa, Artificial sequence
  Synthesized polypeptide
AQTVTQSQPEMSVQEAETVTLSCTYDTSESDYYLFWYKQPPSRQMILVIRQEAYKQQNATENRFSVNFQKAAKSFSLKISDSQLGDAAMYFCAYRSGIIQGAQKLVFGQGTRLTINPNIQNPDPAVYQLRDSKSSDKSVCLFTDFDSQTNVSQSKDSDVYITDKTVLDMRSMDFKSNSAVAWSNKSDFACANAFNNSIIPEDTFFPSPESSCDVKLVEKSFETDTNLNFQNLSVIGFRILLLKVAGFNLLMTLRLWSS

SEQ ID NO: 4 - DNA, 777 bp, Artificial sequence
  Synthesized polynucleotide
gctcagacagtcactcagtctcaaccagagatgtctgtgcaggaggcagagaccgtgaccctgagctgcacatatgacaccagtgagagtgattattatttattctggtacaagcagcctcccagcaggcagatgattctcgttattcgccaagaagcttataagcaacagaatgcaacagagaatcgtttctctgtgaacttccagaaagcagccaaatccttcagtctcaagatctcagactcacagctgggggatgccgcgatgtatttctgtgcttataggagcggcataattcagggagcccagaagctggtatttggccaaggaaccaggctgactatcaacccaaatatccagaaccctgaccctgccgtgtaccagctgagagactctaaatccagtgacaagtctgtctgcctattcaccgattttgattctcaaacaaatgtgtcacaaagtaaggattctgatgtgtatatcacagacaaaactgtgctagacatgaggtctatggacttcaagagcaacagtgctgtggcctggagcaacaaatctgactttgcatgtgcaaacgccttcaacaacagcattattccagaagacaccttcttccccagcccagaaagttcctgtgatgtcaagctggtcgagaaaagctttgaaacagatacgaacctaaactttcaaaacctgtcagtgattgggttccgaatcctcctcctgaaagtggccgggtttaatctgctcatgacgctgcggctgtggtccagctaa

SEQ ID NO: 5 - protein, 116 aa, Artificial sequence
  Synthesized polypeptide
AAGVIQSPRHLIKEKRETATLKCYPIPRHDTVYWYQQGPGQDPQFLISFYEKMQSDKGSIPDRFSAQQFSDYHSELNMSSLELGDSALYFCASSSDRELLFYNEQFFGPGTRLTVL

SEQ ID NO: 6 - DNA, 348 bp, Artificial sequence
  Synthesized polynucleotide
gctgctggagtcatccagtccccaagacatctgatcaaagaaaagagggaaacagccactctgaaatgctatcctatccctagacacgacactgtctactggtaccagcagggtccaggtcaggacccccagttcctcatttcgttttatgaaaagatgcagagcgataaaggaagcatccctgatcgattctcagctcaacagttcagtgactatcattctgaactgaacatgagctccttggagctgggggactcagccctgtacttctgtgccagcagctcagacagggaactattattctacaatgagcagttcttcgggccagggacacggctcaccgtgcta

SEQ ID NO: 7 - protein, 295 aa, Artificial sequence
  Synthesized polypeptide
AAGVIQSPRHLIKEKRETATLKCYPIPRHDTVYWYQQGPGQDPQFLISFYEKMQSDKGSIPDRFSAQQFSDYHSELNMSSLELGDSALYFCASSSDRELLFYNEQFFGPGTRLTVLEDLKNVFPPEVAVFEPSEAEISHTQKATLVCLATGFYPDHVELSWWVNGKEVHSGVSTDPQPLKEQPALNDSRYCLSSRLRVSATFWQNPRNHFRCQVQFYGLSENDEWTQDRAKPVTQIVSAEAWGRADCGFTSESYQQGVLSATILYEILLGKATLYAVLVSALVLMAMVKRKDSRG

SEQ ID NO: 8 - DNA, 888 bp, Artificial sequence
  Synthesized polynucleotide
gctgctggagtcatccagtccccaagacatctgatcaaagaaaagagggaaacagccactctgaaatgctatcctatccctagacacgacactgtctactggtaccagcagggtccaggtcaggacccccagttcctcatttcgttttatgaaaagatgcagagcgataaaggaagcatccctgatcgattctcagctcaacagttcagtgactatcattctgaactgaacatgagctccttggagctgggggactcagccctgtacttctgtgccagcagctcagacagggaactattattctacaatgagcagttcttcgggccagggacacggctcaccgtgctagaggacctgaaaaacgtgttcccacccgaggtcgctgtgtttgagccatcagaagcagagatctcccacacccaaaaggccacactggtgtgcctggccacaggcttctaccccgaccacgtggagctgagctggtgggtgaatgggaaggaggtgcacagtggggtcagcacagacccgcagcccctcaaggagcagcccgccctcaatgactccagatactgcctgagcagccgcctgagggtctcggccaccttctggcagaacccccgcaaccacttccgctgtcaagtccagttctacgggctctcggagaatgacgagtggacccaggatagggccaaacctgtcacccagatcgtcagcgccgaggcctggggtagagcagactgtggcttcacctccgagtcttaccagcaaggggtcctgtctgccaccatcctctatgagatcttgctagggaaggccaccttgtatgccgtgctggtcagtgccctcgtgctgatggccatggtcaagagaaaggattccagaggctaa

SEQ ID NO: 9 - protein, 9 aa, Artificial sequence
  Synthesized polypeptide
KASEKIFYV

SEQ ID NO: 10 - protein, 7 aa, Artificial sequence
  Synthesized polypeptide
TSESDYY

SEQ ID NO: 11 - protein, 8 aa, Artificial sequence
  Synthesized polypeptide
QEAYKQQN

SEQ ID NO: 12 - protein, 14 aa, Artificial sequence
  Synthesized polypeptide
AYRSGIIQGAQKLV

SEQ ID NO: 13 - protein, 5 aa, Artificial sequence
  Synthesized polypeptide
PRHDT

SEQ ID NO: 14 - protein, 6 aa, Artificial sequence
  Synthesized polypeptide
FYEKMQ

SEQ ID NO: 15 - protein, 15 aa, Artificial sequence
  Synthesized polypeptide
ASSSDRELLFYNEQF

SEQ ID NO: 16 - DNA, 21 bp, Artificial sequence
  Synthesized polynucleotide
accagtgagagtgattattat

SEQ ID NO: 17 - DNA, 24 bp, Artificial sequence
  Synthesized polynucleotide
caagaagcttataagcaacagaat

SEQ ID NO: 18 - DNA, 42 bp, Artificial sequence
  Synthesized polynucleotide
gcttataggagcggcataattcagggagcccagaagctggta

SEQ ID NO: 19 - DNA, 15 bp, Artificial sequence
  Synthesized polynucleotide
cctagacacgacact

SEQ ID NO: 20 - DNA, 18 bp, Artificial sequence
  Synthesized polynucleotide
ttttatgaaaagatgcag

SEQ ID NO: 21 - DNA, 45 bp, Artificial sequence
  Synthesized polynucleotide
gccagcagctcagacagggaactattattctacaatgagcagttc

SEQ ID NO: 22 - protein, 278 aa, Artificial sequence
  Synthesized polypeptide
MACPGFLWALVISTCLEFSMAQTVTQSQPEMSVQEAETVTLSCTYDTSESDYYLFWYKQPPSRQMILVIRQEAYKQQNATENRFSVNFQKAAKSFSLKISDSQLGDAAMYFCAYRSGIIQGAQKLVFGQGTRLTINPNIQNPDPAVYQLRDSKSSDKSVCLFTDFDSQTNVSQSKDSDVYITDKTVLDMRSMDFKSNSAVAWSNKSDFACANAFNNSIIPEDTFFPSPESSCDVKLVEKSFETDTNLNFQNLSVIGFRILLLKVAGFNLLMTLRLWSS

SEQ ID NO: 23 - DNA, 837 bp, Artificial sequence
  Synthesized polynucleotide
atggcatgccctggcttcctgtgggcacttgtgatctccacctgtcttgaatttagcatggctcagacagtcactcagtctcaaccagagatgtctgtgcaggaggcagagaccgtgaccctgagctgcacatatgacaccagtgagagtgattattatttattctggtacaagcagcctcccagcaggcagatgattctcgttattcgccaagaagcttataagcaacagaatgcaacagagaatcgtttctctgtgaacttccagaaagcagccaaatccttcagtctcaagatctcagactcacagctgggggatgccgcgatgtatttctgtgcttataggagcggcataattcagggagcccagaagctggtatttggccaaggaaccaggctgactatcaacccaaatatccagaaccctgaccctgccgtgtaccagctgagagactctaaatccagtgacaagtctgtctgcctattcaccgattttgattctcaaacaaatgtgtcacaaagtaaggattctgatgtgtatatcacagacaaaactgtgctagacatgaggtctatggacttcaagagcaacagtgctgtggcctggagcaacaaatctgactttgcatgtgcaaacgccttcaacaacagcattattccagaagacaccttcttccccagcccagaaagttcctgtgatgtcaagctggtcgagaaaagctttgaaacagatacgaacctaaactttcaaaacctgtcagtgattgggttccgaatcctcctcctgaaagtggccgggtttaatctgctcatgacgctgcggctgtggtccagctaa

SEQ ID NO: 24 - protein, 324 aa, Artificial sequence
  Synthesized polypeptide
MLSPDLPDSAWNTRLLCRVMLCLLGAGSVAAGVIQSPRHLIKEKRETATLKCYPIPRHDTVYWYQQGPGQDPQFLISFYEKMQSDKGSIPDRFSAQQFSDYHSELNMSSLELGDSALYFCASSSDRELLFYNEQFFGPGTRLTVLEDLKNVFPPEVAVFEPSEAEISHTQKATLVCLATGFYPDHVELSWWVNGKEVHSGVSTDPQPLKEQPALNDSRYCLSSRLRVSATFWQNPRNHFRCQVQFYGLSENDEWTQDRAKPVTQIVSAEAWGRADCGFTSESYQQGVLSATILYEILLGKATLYAVLVSALVLMAMVKRKDSRG

SEQ ID NO: 25 - DNA, 975 bp, Artificial sequence
  Synthesized polynucleotide
atgcttagtcctgacctgcctgactctgcctggaacaccaggctcctctgccgtgtcatgctttgtctcctgggagcaggttcagtggctgctggagtcatccagtccccaagacatctgatcaaagaaaagagggaaacagccactctgaaatgctatcctatccctagacacgacactgtctactggtaccagcagggtccaggtcaggacccccagttcctcatttcgttttatgaaaagatgcagagcgataaaggaagcatccctgatcgattctcagctcaacagttcagtgactatcattctgaactgaacatgagctccttggagctgggggactcagccctgtacttctgtgccagcagctcagacagggaactattattctacaatgagcagttcttcgggccagggacacggctcaccgtgctagaggacctgaaaaacgtgttcccacccgaggtcgctgtgtttgagccatcagaagcagagatctcccacacccaaaaggccacactggtgtgcctggccacaggcttctaccccgaccacgtggagctgagctggtgggtgaatgggaaggaggtgcacagtggggtcagcacagacccgcagcccctcaaggagcagcccgccctcaatgactccagatactgcctgagcagccgcctgagggtctcggccaccttctggcagaacccccgcaaccacttccgctgtcaagtccagttctacgggctctcggagaatgacgagtggacccaggatagggccaaacctgtcacccagatcgtcagcgccgaggcctggggtagagcagactgtggcttcacctccgagtcttaccagcaaggggtcctgtctgccaccatcctctatgagatcttgctagggaaggccaccttgtatgccgtgctggtcagtgccctcgtgctgatggccatggtcaagagaaaggattccagaggctaa

SEQ ID NO: 26 - protein, 212 aa, Artificial sequence
  Synthesized polypeptide
MAQTVTQSQPEMSVQEAETVTLSCTYDTSESDYYLFWYKQPPSRQMILVIRQEAYKQQNATENRFSVNFQKAAKSFSLKISDSQLGDAAMYFCAYRSGIIQGAQKLVFGQGTRLTINPNIQNPDPAVYQLRDSKSSDKSVCLFTDFDSQTNVSQSKDSDVYITDKCVLDMRSMDFKSNSAVAWSNKSDFACANAFNNSIIPEDTFFPSPESS

SEQ ID NO: 27 - DNA, 636 bp, Artificial sequence
  Synthesized polynucleotide
atggcgcagaccgtgacccagtctcaaccagagatgtctgtgcaggaggcagagaccgtgaccctgagctgcacatatgacaccagtgagagtgattattatttattctggtacaagcagcctcccagcaggcagatgattctcgttattcgccaagaagcttataagcaacagaatgcaacagagaatcgtttctctgtgaacttccagaaagcagccaaatccttcagtctcaagatctcagactcacagctgggggatgccgcgatgtatttctgtgcttataggagcggcataattcagggagcccagaagctggtatttggccaaggaaccaggctgactatcaacccaaatatccagaaccctgaccctgccgtgtaccagctgagagactctaagtcgagtgacaagtctgtctgcctattcaccgattttgattctcaaacaaatgtgtcacaaagtaaggattctgatgtgtatatcacagacaaatgtgtgctagacatgaggtctatggacttcaagagcaacagtgctgtggcctggagcaacaaatctgactttgcatgtgcaaacgccttcaacaacagcattattccagaagacaccttcttccccagcccagaaagttcc

SEQ ID NO: 28 - protein, 247 aa, Artificial sequence
  Synthesized polypeptide
MAAGVIQSPRHLIKEKRETATLKCYPIPRHDTVYWYQQGPGQDPQFLISFYEKMQSDKGSIPDRFSAQQFSDYHSELNMSSLELGDSALYFCASSSDRELLFYNEQFFGPGTRLTVLEDLKNVFPPEVAVFEPSEAEISHTQKATLVCLATGFYPDHVELSWWVNGKEVHSGVCTDPQPLKEQPALNDSRYALSSRLRVSATFWQDPRNHFRCQVQFYGLSENDEWTQDRAKPVTQIVSAEAWGRAD

SEQ ID NO: 29 - DNA, 741 bp, Artificial sequence
  Synthesized polynucleotide
atggcggcgggcgtgattcagtccccaagacatctgatcaaagaaaagagggaaacagccactctgaaatgctatcctatccctagacacgacactgtctactggtaccagcagggtccaggtcaggacccccagttcctcatttcgttttatgaaaagatgcagagcgataaaggaagcatccctgatcgattctcagctcaacagttcagtgactatcattctgaactgaacatgagctccttggagctgggggactcagccctgtacttctgtgccagcagctcagacagggaactattattctacaatgagcagttcttcgggccagggacacggctcaccgtgctagaggacctgaaaaacgtgttcccacccgaggtcgctgtgtttgagccatcagaagcagagatctcccacacccaaaaggccacactggtgtgcctggccaccggtttctaccccgaccacgtggagctgagctggtgggtgaatgggaaggaggtgcacagtggggtctgcacagacccgcagcccctcaaggagcagcccgccctcaatgactccagatacgctctgagcagccgcctgagggtctcggccaccttctggcaggacccccgcaaccacttccgctgtcaagtccagttctacgggctctcggagaatgacgagtggacccaggatagggccaaacccgtcacccagatcgtcagcgccgaggcctggggtagagcagac

SEQ ID NO: 30 - protein, 258 aa, Artificial sequence
  Synthesized polypeptide
MAQTVTQSQPELSVQEGETVTISCTYDTSESDYYLFWYKQPPSRQPILVIRQEAYKQQNATENRFSVNFQKAAKSFSLKISDVQPGDAAMYFCAYRSGIIQGAQKLVFGQGTRLTINPGGGSEGGGSEGGGSEGGGSEGGTGAAGVTQSPRHLSVEKGETVTLKCYPIPRHDTVYWYQQGPGQDLQFLISFYEKMQSDKGSIPDRFSAQQFSDYHSELNISSVEPGDSALYFCASSSDRELLFYNEQFFGPGTRLTVD

SEQ ID NO: 31 - DNA, 774 bp, Artificial sequence
  Synthesized polynucleotide
atggctcaaactgttactcagagccaaccggagctgagcgtgcaagagggtgaaaccgttaccatcagctgcacctacgacaccagcgaaagcgattactacctgttctggtataagcagccgccgagccgtcaaccgatcctggttattcgtcaggaagcgtacaaacagcaaaacgcgaccgaaaaccgtttcagcgtgaactttcagaaggcggcgaaaagcttcagcctgaagatcagcgacgttcaaccgggcgatgcggcgatgtacttttgcgcgtatcgtagcggtatcattcagggcgcgcaaaaactggtgttcggtcagggcacccgtctgaccattaacccgggtggcggtagcgagggcggtggcagcgaaggtggcggtagcgagggcggtggcagcgaaggtggcaccggtgcggcgggcgtgacccaaagcccgcgtcacctgagcgtggagaagggtgaaaccgttaccctgaaatgctatccgatcccgcgtcacgacaccgtttactggtatcagcaaggtccgggccaggatctgcaattcctgatcagcttttacgagaagatgcagagcgacaaaggtagcattccggatcgtttcagcgcgcagcaatttagcgactatcacagcgagctgaacattagcagcgtggaaccgggtgacagcgcgctgtacttctgcgcgagcagcagcgatcgtgagctgctgttttataacgaacagttctttggtccgggcacccgtctgaccgttgat

SEQ ID NO: 32 - protein, 118 aa, Artificial sequence
  Synthesized polypeptide
MAQTVTQSQPELSVQEGETVTISCTYDTSESDYYLFWYKQPPSRQPILVIRQEAYKQQNATENRFSVNFQKAAKSFSLKISDVQPGDAAMYFCAYRSGIIQGAQKLVFGQGTRLTINP

SEQ ID NO: 33 - DNA, 354 bp, Artificial sequence
  Synthesized polynucleotide
atggctcaaactgttactcagagccaaccggagctgagcgtgcaagagggtgaaaccgttaccatcagctgcacctacgacaccagcgaaagcgattactacctgttctggtataagcagccgccgagccgtcaaccgatcctggttattcgtcaggaagcgtacaaacagcaaaacgcgaccgaaaaccgtttcagcgtgaactttcagaaggcggcgaaaagcttcagcctgaagatcagcgacgttcaaccgggcgatgcggcgatgtacttttgcgcgtatcgtagcggtatcattcagggcgcgcaaaaactggtgttcggtcagggcacccgtctgaccattaacccg

SEQ ID NO: 34 - protein, 116 aa, Artificial sequence
  Synthesized polypeptide
AAGVTQSPRHLSVEKGETVTLKCYPIPRHDTVYWYQQGPGQDLQFLISFYEKMQSDKGSIPDRFSAQQFSDYHSELNISSVEPGDSALYFCASSSDRELLFYNEQFFGPGTRLTVD

SEQ ID NO: 35 - DNA, 348 bp, Artificial sequence
  Synthesized polynucleotide
gcggcgggcgtgacccaaagcccgcgtcacctgagcgtggagaagggtgaaaccgttaccctgaaatgctatccgatcccgcgtcacgacaccgtttactggtatcagcaaggtccgggccaggatctgcaattcctgatcagcttttacgagaagatgcagagcgacaaaggtagcattccggatcgtttcagcgcgcagcaatttagcgactatcacagcgagctgaacattagcagcgtggaaccgggtgacagcgcgctgtacttctgcgcgagcagcagcgatcgtgagctgctgttttataacgaacagttctttggtccgggcacccgtctgaccgttgat

SEQ ID NO: 36 - protein, 24 aa, Artificial sequence
  Synthesized polypeptide
GGGSEGGGSEGGGSEGGGSEGGTG

SEQ ID NO: 37 - DNA, 72 bp, Artificial sequence
  Synthesized polynucleotide
ggtggcggtagcgagggcggtggcagcgaaggtggcggtagcgagggcggtggcagcgaaggtggcaccggt